European Patent Application EP 4 249 472 A2, published September 27, 2023. Title: METHODS FOR MODULATING RNA SPLICING. Applicant: PTC Therapeutics, Inc. The sequence listing filed with the application follows.

SEQUENCE LISTING (120 sequences)

SEQ ID NO: 1-9 - skipped (9 entries)

SEQ ID NO: 10 - DNA, 28 bp, synthetic construct
  source 1..28: mol_type = other DNA; note = Forward primer used for preparing SNM2 minigene construct
cgcggatccataattcccccaccacctc

SEQ ID NO: 11 - DNA, 28 bp, synthetic construct
  source 1..28: mol_type = other DNA; note = Reverse primer used for preparing SNM2 minigene construct
cgcggatccgtgctgctctatgccagca

SEQ ID NO: 12 - DNA, 21 bp, synthetic construct
  source 1..21: mol_type = other DNA; note = Forward primer used for amplifying only transcripts derived from the transfected plasmids
gatgctgatgctttgggaagt

SEQ ID NO: 13 - DNA, 19 bp, synthetic construct
  source 1..19: mol_type = other DNA; note = primer used for identifying alternatively spliced mRNAs -APLP2e6F1
acggcaccatgtcagacaa

SEQ ID NO: 14 - DNA, 20 bp, synthetic construct
  source 1..20: mol_type = other DNA; note = Primer used for identifying alternatively spliced mRNAs - APLP2e8R1
caacatcattggttggcaga

SEQ ID NO: 15 - DNA, 21 bp, synthetic construct
  source 1..21: mol_type = other DNA; note = Primer used for identifying alternatively spliced mRNAs - STRN3e7F1
actgctgaagatggtgaagga

SEQ ID NO: 16 - DNA, 23 bp, synthetic construct
  source 1..23: mol_type = other DNA; note = Primer used for identifying alternatively spliced mRNAs - STRN3e9R1
ccagatcagctatcatgtcgtag

SEQ ID NO: 17 - DNA, 19 bp, synthetic construct
  source 1..19: mol_type = other DNA; note = Primer used for identifying alternatively spliced mRNAs - RCC1e3F1
agacgatctgcacttcgca

SEQ ID NO: 18 - DNA, 21 bp, synthetic construct
  source 1..21: mol_type = other DNA; note = Primer used for identifying alternatively spliced mRNAs - RCC1e5e6R1
gtgagaccttcaccttcttgc

SEQ ID NO: 19 - DNA, 23 bp, synthetic construct
  source 1..23: mol_type = other DNA; note = Primer used for identifying alternatively spliced mRNAs - ERGIC3e6F1
tgtatggcttcttggaagtcaat

SEQ ID NO: 20 - DNA, 24 bp, synthetic construct
  source 1..24: mol_type = other DNA; note = Primer used for identifying alternatively spliced mRNAs - ERGIC3e9e10R1
gtagtgggtcatgttgatgttgtc

SEQ ID NO: 21 - DNA, 22 bp, synthetic construct
  source 1..22: mol_type = other DNA; note = Primer used for identifying alternatively spliced mRNAs - SMN Rev
cgcttcacattccagatctgtc

SEQ ID NO: 22 - DNA, 17 bp, synthetic construct
  source 1..17: mol_type = other DNA; note = Primer used for identifying alternatively spliced mRNAs - FOXM1 For
gtgttgcagccctcggt

SEQ ID NO: 23 - DNA, 21 bp, synthetic construct
  source 1..21: mol_type = other DNA; note = Primer used for identifying alternatively spliced mRNAs - FOXM1 Rev
tgaactggaagcaaaggagaa

SEQ ID NO: 24 - DNA, 18 bp, synthetic construct
  source 1..18: mol_type = other DNA; note = Primer used for identifying alternatively spliced mRNAs - VPS29e1F1
cggtggtggtgactgagc

SEQ ID NO: 25 - DNA, 21 bp, synthetic construct
  source 1..21: mol_type = other DNA; note = Primer used for identifying alternatively spliced mRNAs - VPS29e3R1
gggatgtgcagatctcctaat

SEQ ID NO: 26 - DNA, 26 bp, synthetic construct
  source 1..26: mol_type = other DNA; note = Primer used for identifying alternatively spliced mRNAs - GGCTe1F1
agatgaggagagttttctgtactttg

SEQ ID NO: 27 - DNA, 20 bp, synthetic construct
  source 1..20: mol_type = other DNA; note = Primer used for identifying alternatively spliced mRNAs - GGCTe4R1
tctcttgatactccagcggc

SEQ ID NO: 28 - DNA, 23 bp, synthetic construct
  source 1..23: mol_type = other DNA; note = Primer used for identifying alternatively spliced mRNAs - PRKDC e9F1
gatctgaagagatatgctgtgcc

SEQ ID NO: 29 - DNA, 20 bp, synthetic construct
  source 1..20: mol_type = other DNA; note = Primer used for identifying alternatively spliced mRNAs - PRKDC e12R1
acggtcgtcaccagtgtctg

SEQ ID NO: 30 - DNA, 23 bp, synthetic construct
  source 1..23: mol_type = other DNA; note = Primer used for identifying alternatively spliced mRNAs - PRKDC e50F1
gggtccctaaagatgaagtgtta

SEQ ID NO: 31 - DNA, 22 bp, synthetic construct
  source 1..22: mol_type = other DNA; note = Primer used for identifying alternatively spliced mRNAs - PRKDC e52R1
attcaccaaagcctggaagtat

SEQ ID NO: 32 - DNA, 24 bp, synthetic construct
  source 1..24: mol_type = other DNA; note = Primer used for identifying alternatively spliced mRNAs - MADD e20F1
cagaaagtgtaaataccccagttg

SEQ ID NO: 33 - DNA, 19 bp, synthetic construct
  source 1..19: mol_type = other DNA; note = Primer used for identifying alternatively spliced mRNAs - MADD e22R1
gctcacaccactgtctgcg

SEQ ID NO: 34 - DNA, 22 bp, synthetic construct
  source 1..22: mol_type = other DNA; note = Primer used for identifying alternatively spliced mRNAs - LARP7 5'UTRF1
cttccttggcttcgagtctctc

SEQ ID NO: 35 - DNA, 25 bp, synthetic construct
  source 1..25: mol_type = other DNA; note = Primer used for identifying alternatively spliced mRNAs - LARP7 e2R1
cctgtgtcctatcatttgttttctc

SEQ ID NO: 36 - DNA, 23 bp, synthetic construct
  source 1..23: mol_type = other DNA; note = Primer used for identifying alternatively spliced mRNAs - LARP7 e1F1
cgaaagtaaccgagactatcagg

SEQ ID NO: 37 - DNA, 22 bp, synthetic construct
  source 1..22: mol_type = other DNA; note = Primer used for identifying alternatively spliced mRNAs - LARP7 e4R1
ttcagtgctttcttcttccatt

SEQ ID NO: 38 - DNA, 19 bp, synthetic construct
  source 1..19: mol_type = other DNA; note = Primer used for identifying alternatively spliced mRNAs - ARMCX6 e2F1
cggcacaagtttcagcgag

SEQ ID NO: 39 - DNA, 22 bp, synthetic construct
  source 1..22: mol_type = other DNA; note = Primer used for identifying alternatively spliced mRNAs - ARMCX6 e4R1
cagggtgagtaaggatggaggg

SEQ ID NO: 40 - DNA, 21 bp, synthetic construct
  source 1..21: mol_type = other DNA; note = Primer used for identifying alternatively spliced mRNAs - GALC e4F1
ggatacgagtggtggttgatg

SEQ ID NO: 41 - DNA, 23 bp, synthetic construct
  source 1..23: mol_type = other DNA; note = Primer used for identifying alternatively spliced mRNAs - GALC e7R1
cagagatggactcccagagatta

SEQ ID NO: 42 - DNA, 20 bp, synthetic construct
  source 1..20: mol_type = other DNA; note = Primer used for identifying alternatively spliced mRNAs - LAMA2 e4F1
ggattttggaacgctctctt

SEQ ID NO: 43 - DNA, 26 bp, synthetic construct
  source 1..26: mol_type = other DNA; note = Primer used for identifying alternatively spliced mRNAs - LAMA2 e6R1
gaaatatccttgaccgagtagtaata

SEQ ID NO: 44 - DNA, 22 bp, synthetic construct
  source 1..22: mol_type = other DNA; note = Primer used for identifying alternatively spliced mRNAs - ABHD10e4F1
gagaaggtcgtggctcttattg

SEQ ID NO: 45 - DNA, 23 bp, synthetic construct
  source 1..23: mol_type = other DNA; note = Primer used for identifying alternatively spliced mRNAs - ABHD10e6R1
gggctatgtaacaagcagtgatg

SEQ ID NO: 46 - DNA, 19 bp, synthetic construct
  source 1..19: mol_type = other DNA; note = Primer used for identifying alternatively spliced mRNAs - FADS2e5F1
ctgccaactggtggaatca

SEQ ID NO: 47 - DNA, 22 bp, synthetic construct
  source 1..22: mol_type = other DNA; note = Primer used for identifying alternatively spliced mRNAs - FADS2e8R1
gatgccgtagaaagggatgtag

SEQ ID NO: 48 - DNA, 21 bp, synthetic construct
  source 1..21: mol_type = other DNA; note = Primer used for identifying alternatively spliced mRNAs - DIAPH3e10F1
tcaatgccctggttacatctc

SEQ ID NO: 49 - DNA, 24 bp, synthetic construct
  source 1..24: mol_type = other DNA; note = Primer used for identifying alternatively spliced mRNAs - DIAPH3e13R1
acaatctgggatacacactcatca

SEQ ID NO: 50 - DNA, 24 bp, synthetic construct
  source 1..24: mol_type = other DNA; note = Primer used for identifying alternatively spliced mRNAs - PDIA3e3F1
ctgccaacactaacacctgtaata

SEQ ID NO: 51 - DNA, 22 bp, synthetic construct
  source 1..22: mol_type = other DNA; note = Primer used for identifying alternatively spliced mRNAs - PDIA3e7R1
agtccttgccctgtatcaaatc

SEQ ID NO: 52 - DNA, 21 bp, synthetic construct
  source 1..21: mol_type = other DNA; note = Primer used for identifying alternatively spliced mRNAs - FN1e34F1
gctcatccgtggttgtatcag

SEQ ID NO: 53 - DNA, 23 bp, synthetic construct
  source 1..23: mol_type = other DNA; note = Primer used for identifying alternatively spliced mRNAs - FN1e36R1
gatcgtctcagtcttggttctcc

SEQ ID NO: 54 - DNA, 21 bp, synthetic construct
  source 1..21: mol_type = other DNA; note = Primer used for identifying alternatively spliced mRNAs - PARP1e20F1
agtgccaactactgccatacg

SEQ ID NO: 55 - DNA, 23 bp, synthetic construct
  source 1..23: mol_type = other DNA; note = Primer used for identifying alternatively spliced mRNAs - PARP1ee23R1
aatcctttctgaggtggtttagt

SEQ ID NO: 56 - DNA, 20 bp, synthetic construct
  source 1..20: mol_type = other DNA; note = Primer used for identifying alternatively spliced mRNAs - COL1Ae2F1
caaggtgttgtgcgatgacg

SEQ ID NO: 57 - DNA, 26 bp, synthetic construct
  source 1..26: mol_type = other DNA; note = Primer used for identifying alternatively spliced mRNAs - COL1Ae6R1
ggttgatttctcatcatagccataag

SEQ ID NO: 58 - DNA, 20 bp, synthetic construct
  source 1..20: mol_type = other DNA; note = Primer used for identifying alternatively spliced mRNAs - COLA1e7F1
cctctggtcctcgtggtctc

SEQ ID NO: 59 - DNA, 20 bp, synthetic construct
  source 1..20: mol_type = other DNA; note = Primer used for identifying alternatively spliced mRNAs - COL1Ae12R1
ccatccaaaccactgaaacc

SEQ ID NO: 60 - DNA, 19 bp, synthetic construct
  source 1..19: mol_type = other DNA; note = Primer used for identifying alternatively spliced mRNAs - COLA1e27F1
ggtcctgctggcaaagatg

SEQ ID NO: 61 - DNA, 18 bp, synthetic construct
  source 1..18: mol_type = other DNA; note = Primer used for identifying alternatively spliced mRNAs - COLA1e31R1
gctcgccagggaaacctc

SEQ ID NO: 62 - DNA, 19 bp, synthetic construct
  source 1..19: mol_type = other DNA; note = Primer used for identifying alternatively spliced mRNAs - COLA1e31F1
aggcgagagaggtttccct

SEQ ID NO: 63 - DNA, 21 bp, synthetic construct
  source 1..21: mol_type = other DNA; note = Primer used for identifying alternatively spliced mRNAs - COLA1e33e34R1
ggaccactttcacccttgtca

SEQ ID NO: 64 - DNA, 19 bp, synthetic construct
  source 1..19: mol_type = other DNA; note = Primer used for identifying alternatively spliced mRNAs - COLA1e47F1
gggcgacagaggcataaag

SEQ ID NO: 65 - DNA, 20 bp, synthetic construct
  source 1..20: mol_type = other DNA; note = Primer used for identifying alternatively spliced mRNAs - COLA1e48R1
tcacggtcacgaaccacatt

SEQ ID NO: 66 - DNA, 22 bp, synthetic construct
  source 1..22: mol_type = other DNA; note = Primer used for identifying alternatively spliced mRNAs - COL1A2e20F1
caaaggagagagcggtaacaag

SEQ ID NO: 67 - DNA, 22 bp, synthetic construct
  source 1..22: mol_type = other DNA; note = Primer used for identifying alternatively spliced mRNAs - COL1A2e22R1
aagaccacgagaaccaggacta

SEQ ID NO: 68 - DNA, 19 bp, synthetic construct
  source 1..19: mol_type = other DNA; note = Primer used for identifying alternatively spliced mRNAs - COL1A2e22F1
cctggttctcgtggtcttc

SEQ ID NO: 69 - DNA, 18 bp, synthetic construct
  source 1..18: mol_type = other DNA; note = Primer used for identifying alternatively spliced mRNAs - COL1A2e24e25R1
gccgacaggaccttcttt

SEQ ID NO: 70 - DNA, 19 bp, synthetic construct
  source 1..19: mol_type = other DNA; note = Primer used for identifying alternatively spliced mRNAs - COL1A2e29F1
tggcaaaccaggagaaagg

SEQ ID NO: 71 - DNA, 20 bp, synthetic construct
  source 1..20: mol_type = other DNA; note = Primer used for identifying alternatively spliced mRNAs - COL1A2e31R1
aaggacctcggcttccaata

SEQ ID NO: 72 - DNA, 18 bp, synthetic construct
  source 1..18: mol_type = other DNA; note = Primer used for identifying alternatively spliced mRNAs - COL3A1e7e8F1
ggcaagctggtccttcag

SEQ ID NO: 73 - DNA, 19 bp, synthetic construct
  source 1..19: mol_type = other DNA; note = Primer used for identifying alternatively spliced mRNAs - COL3A1e11R1
ggagcacctgtttcaccct

SEQ ID NO: 74 - DNA, 23 bp, synthetic construct
  source 1..23: mol_type = other DNA; note = Primer used for identifying alternatively spliced mRNAs - COL3A1e45F1
tgacaaaggtgaaacaggtgaac

SEQ ID NO: 75 - DNA, 20 bp, synthetic construct
  source 1..20: mol_type = other DNA; note = Primer used for identifying alternatively spliced mRNAs - COL3A1e47R1
gtccactgggtccaacaggt

SEQ ID NO: 76 - DNA, 20 bp, synthetic construct
  source 1..20: mol_type = other DNA; note = Primer used for identifying alternatively spliced mRNAs - COL5A2e10e11F1
aatgggtccgattggttcac

SEQ ID NO: 77 - DNA, 22 bp, synthetic construct
  source 1..22: mol_type = other DNA; note = Primer used for identifying alternatively spliced mRNAs - COL52Ae16R1
caagtctccctctctctcctgg

SEQ ID NO: 78 - DNA, 21 bp, synthetic construct
  source 1..21: mol_type = other DNA; note = Primer used for identifying alternatively spliced mRNAs - COL52Ae30F1
ggtgaaagaggagaacaagga

SEQ ID NO: 79 - DNA, 20 bp, synthetic construct
  source 1..20: mol_type = other DNA; note = Primer used for identifying alternatively spliced mRNAs - COL52Ae33R1
tcaccagggagtccagttat

SEQ ID NO: 80 - DNA, 22 bp, synthetic construct
  source 1..22: mol_type = other DNA; note = Primer used for identifying alternatively spliced mRNAs - COL52Ae33F1
agaacctgggataactggactc

SEQ ID NO: 81 - DNA, 21 bp, synthetic construct
  source 1..21: mol_type = other DNA; note = Primer used for identifying alternatively spliced mRNAs - COL5A2e35e36R1
agacctcttgcaccatcattt

SEQ ID NO: 82 - DNA, 17 bp, synthetic construct
  source 1..17: mol_type = other DNA; note = Primer used for identifying alternatively spliced mRNAs - COL5A2e33F1
agggaatggctggagga

SEQ ID NO: 83 - DNA, 19 bp, synthetic construct
  source 1..19: mol_type = other DNA; note = Primer used for identifying alternatively spliced mRNAs - COL5A2e36R1
cccaaaggacctggaagac

SEQ ID NO: 84 - DNA, 20 bp, synthetic construct
  source 1..20: mol_type = other DNA; note = Primer used for identifying alternatively spliced mRNAs - COL5A2e48F1
aggacctcgtggtgacaaag

SEQ ID NO: 85 - DNA, 20 bp, synthetic construct
  source 1..20: mol_type = other DNA; note = Primer used for identifying alternatively spliced mRNAs - COL5A2e50R1
gcccagggtttccttcttta

SEQ ID NO: 86 - DNA, 23 bp, synthetic construct
  source 1..23: mol_type = other DNA; note = Primer used for identifying alternatively spliced mRNAs - SMNe4F1
gatgaaagtgagaactccaggtc

SEQ ID NO: 87 - DNA, 21 bp, synthetic construct
  source 1..21: mol_type = other DNA; note = Primer used for identifying alternatively spliced mRNAs - SMNe6R1
caaagcatcagcatcatcaag

SEQ ID NO: 88 - RNA, 10 nt, synthetic construct
  source 1..10: mol_type = other RNA; note = sequence motif resulted in a compound-dependent increase in the inclusion of exon 7 of SMN2
aggagtaagt

SEQ ID NO: 89 - DNA, 10 bp, synthetic construct
  source 1..10: mol_type = other DNA; note = sequence motif resulted in selectivity against the inclusion of exon 7A of FOXM1
atcagtaagt

SEQ ID NO: 90 - DNA, 10 bp, synthetic construct
  source 1..10: mol_type = other DNA; note = Alternative splicing sequence motif which affected exon 7A Delta-C of gene FOXM1, or exon 7 of APLP2
atgagtaagt

SEQ ID NO: 91-95 - skipped (5 entries)

SEQ ID NO: 96 - DNA, 10 bp, synthetic construct
  source 1..10: mol_type = other DNA; note = Alternative splicing sequence motif which affected exon 7 of gene SMN2, or exon 5 of COL1A1
aggagtaagt

SEQ ID NO: 97 - DNA, 10 bp, synthetic construct
  source 1..10: mol_type = other DNA; note = Alternative splicing sequence motif which affected exon 2 of gene GGCT
atgagtaggt

SEQ ID NO: 98 - DNA, 10 bp, synthetic construct
  source 1..10: mol_type = other DNA; note = Alternative splicing sequence motif which affected exon 5 of gene ABHD10
atgagtatgt

SEQ ID NO: 99 - DNA, 10 bp, synthetic construct
  source 1..10: mol_type = other DNA; note = Alternative splicing sequence motif which affected exon 8 of gene STRN3, exon 30 of COL1A1, exon 5 of LAMA2, exon 30 of COL1A2, exon 35 of COL5A2, or exon 49 of COL5A2
aagagtaagt

SEQ ID NO: 100 - DNA, 10 bp, synthetic construct
  source 1..10: mol_type = other DNA; note = Alternative splicing sequence motif which affected exon 2 of gene VPS29, exon 32 of COL1A1, exon 22 of COL1A2, exon 10 of COL3A1, exon 46 of COL3A1, or exon 34 of COL5A2
cagagtaagt

SEQ ID NO: 101 - DNA, 10 bp, synthetic construct
  source 1..10: mol_type = other DNA; note = Alternative splicing sequence motif which affected exon 8 of gene ERGIC3, or exon 35 of FN1
gagagtaagt

SEQ ID NO: 102 - DNA, 10 bp, synthetic construct
  source 1..10: mol_type = other DNA; note = Alternative splicing sequence motif which affected exon 21 of gene MADD
cagagtaagg

SEQ ID NO: 103 - DNA, 10 bp, synthetic construct
  source 1..10: mol_type = other DNA; note = Alternative splicing sequence motif which affected exon 1 of gene LARP7
cggagtaagt

SEQ ID NO: 104 - DNA, 10 bp, synthetic construct
  source 1..10: mol_type = other DNA; note = Alternative splicing sequence motif which affected exon 2 of gene LARP7
aagagtaaga

SEQ ID NO: 105 - DNA, 10 bp, synthetic construct
  source 1..10: mol_type = other DNA; note = Alternative splicing sequence motif which affected exon 3 of gene ARMCX6
tagagtatga

SEQ ID NO: 106 - DNA, 10 bp, synthetic construct
  source 1..10: mol_type = other DNA; note = Alternative splicing sequence motif which affected exon 5 of gene GALC
tggagttagt

SEQ ID NO: 107 - DNA, 10 bp, synthetic construct
  source 1..10: mol_type = other DNA; note = Alternative splicing sequence motif which affected exon 11 of gene PRKDC
aggagtatgt

SEQ ID NO: 108 - DNA, 10 bp, synthetic construct
  source 1..10: mol_type = other DNA; note = Alternative splicing sequence motif which affected exon 51 of gene PRKDC
gcgagtacgt

SEQ ID NO: 109 - DNA, 10 bp, synthetic construct
  source 1..10: mol_type = other DNA; note = Alternative splicing sequence motif which affected exon 4 of gene RCC1
agaggtaaga

SEQ ID NO: 110 - DNA, 10 bp, synthetic construct
  source 1..10: mol_type = other DNA; note = Alternative splicing sequence motif which affected exon 6 of gene FADS2
ctgagtaagt

SEQ ID NO: 111 - DNA, 10 bp, synthetic construct
  source 1..10: mol_type = other DNA; note = Alternative splicing sequence motif which affected exon 11 of gene DIAPH3
ttgaatatcc

SEQ ID NO: 112 - DNA, 10 bp, synthetic construct
  source 1..10: mol_type = other DNA; note = Alternative splicing sequence motif which affected exon 35 of gene PARP1
acgagtatcc

SEQ ID NO: 113 - DNA, 10 bp, synthetic construct
  source 1..10: mol_type = other DNA; note = Alternative splicing sequence motif which affected exon 11 of gene COL1A1
cagagtgagt

SEQ ID NO: 114 - DNA, 10 bp, synthetic construct
  source 1..10: mol_type = other DNA; note = Alternative splicing sequence motif which affected exon 46 of gene COL1A1 or exon 13 of COL5A2
ccgagtaagt

SEQ ID NO: 115 - DNA, 10 bp, synthetic construct
  source 1..10: mol_type = other DNA; note = Alternative splicing sequence motif which affected exon 21 of gene COL1A2
gagagtaggt

SEQ ID NO: 116 - DNA, 10 bp, synthetic construct
  source 1..10: mol_type = other DNA; note = Alternative splicing sequence motif which affected exon 32 of gene COL5A2
tagagtaagt

SEQ ID NO: 117 - DNA, 10 bp, synthetic construct
  source 1..10: mol_type = other DNA; note = Alternative splicing sequence motif which affected exon 5 of gene SMN2
accagtaagt

SEQ ID NO: 118 - RNA, 23 nt, synthetic construct
  source 1..23: mol_type = other RNA; note = TSL2 (terminal stem loop 2) in SMN2
attccttaaattaaggagtaagt

SEQ ID NO: 119 - RNA, 23 nt, synthetic construct
  source 1..23: mol_type = other RNA; note = Sequence illustrating examplary mutations introduced into TSL2 in SMN2
attccataaattatggagtaagt

SEQ ID NO: 120 - skipped